European Patent Application EP 4 563 165 A1, published June 4, 2025. Title: PSMA-STEAP1 DUAL VARIABLE DOMAIN IMMUNOGLOBULIN (DVD-Ig) MOLECULES AND DRUG CONJUGATES. Applicant: AbbVie Inc. The sequence listing filed with the application follows.

SEQUENCE LISTING (28 sequences)

SEQ ID NO: 1 - protein, 583 aa, synthetic construct
EVQLVESGGGVVQPGRSLRLSCVASGFPFNNYWMTWIRQAPGKGLEWIASITITGGTTYYPGSVKGRFTISRDNSKSTLYLQMNSLRAEDTAVYYCTRERYSTEYYPYYWYFDFWGQGTMVTVSSGGGGSGGGGSEVQLVQSGAEVKKPGSSVKVSCKASGYTFTDYYMNWVKQAPGKGLEWIGLINPSNTGTNYNQKFRDKATLTVDKSTSTAYMELSSLRSEDTAVYYCARRAQATSGDYWGQGTTVTVSSASTKGPSVFPLAPSSKSTSGGTAALGCLVKDYFPEPVTVSWNSGALTSGVHTFPAVLQSSGLYSLSSVVTVPSSSLGTQTYICNVNHKPSNTKVDKKVEPKSCDKTHTCPPCPAPEAAGGPSVFLFPPKPKDTLMISRTPEVTCVVVDVSHEDPEVKFNWYVDGVEVHNAKTKPREEQYNSTYRVVSVLTVLHQDWLNGKEYKCKVSNKALPAPIEKTISKAKGQPREPQVYTLPPSREEMTKNQVSLTCLVKGFYPSDIAVEWESNGQPENNYKTTPPVLDSDGSFFLYSKLTVDKSRWQQGNVFSCSVMHEALHNHYTQKSLSLSPGK

SEQ ID NO: 2 - protein, 125 aa, synthetic construct
EVQLVESGGGVVQPGRSLRLSCVASGFPFNNYWMTWIRQAPGKGLEWIASITITGGTTYYPGSVKGRFTISRDNSKSTLYLQMNSLRAEDTAVYYCTRERYSTEYYPYYWYFDFWGQGTMVTVSS

SEQ ID NO: 3 - protein, 10 aa, synthetic construct
GFPFNNYWMT

SEQ ID NO: 4 - protein, 17 aa, synthetic construct
SITITGGTTYYPGSVKG

SEQ ID NO: 5 - protein, 16 aa, synthetic construct
ERYSTEYYPYYWYFDF

SEQ ID NO: 6 - protein, 10 aa, synthetic construct
GGGGSGGGGS

SEQ ID NO: 7 - protein, 118 aa, synthetic construct
EVQLVQSGAEVKKPGSSVKVSCKASGYTFTDYYMNWVKQAPGKGLEWIGLINPSNTGTNYNQKFRDKATLTVDKSTSTAYMELSSLRSEDTAVYYCARRAQATSGDYWGQGTTVTVSS

SEQ ID NO: 8 - protein, 10 aa, synthetic construct
GYTFTDYYMN

SEQ ID NO: 9 - protein, 17 aa, synthetic construct
LINPSNTGTNYNQKFRD

SEQ ID NO: 10 - protein, 9 aa, synthetic construct
RAQATSGDY

SEQ ID NO: 11 - protein, 331 aa, synthetic construct
DIQMTQSPSSLSASVGDRVTITCRTSQDIGNYLRWFQQKPGKSPKLMIYDAINLAAGVPSRFSGSGSGTDYTLTISSLQPEDVATYYCLQHNEYPYTFGQGTKLEIKRGGSGGGGSGDIQMTQSPSSLSASVGDRVTITCHASQNINVWLSWYQQKPGKAPKLLIYKASNLHTGVPSRFSGSGSGTDFTFTISSLQPEDIATYYCQQGQTYPLTFGGGTKVEIKRTVAAPSVFIFPPSDEQLKSGTASVVCLLNNFYPREAKVQWKVDNALQSGNSQESVTEQDSKDSTYSLSSTLTLSKADYEKHKVYACEVTHQGLSSPVTKSFNRGEA

SEQ ID NO: 12 - protein, 107 aa, synthetic construct
DIQMTQSPSSLSASVGDRVTITCRTSQDIGNYLRWFQQKPGKSPKLMIYDAINLAAGVPSRFSGSGSGTDYTLTISSLQPEDVATYYCLQHNEYPYTFGQGTKLEIK

SEQ ID NO: 13 - protein, 11 aa, synthetic construct
RTSQDIGNYLR

SEQ ID NO: 14 - protein, 7 aa, synthetic construct
DAINLAA

SEQ ID NO: 15 - protein, 9 aa, synthetic construct
LQHNEYPYT

SEQ ID NO: 16 - protein, 9 aa, synthetic construct
GGSGGGGSG

SEQ ID NO: 17 - protein, 107 aa, synthetic construct
DIQMTQSPSSLSASVGDRVTITCHASQNINVWLSWYQQKPGKAPKLLIYKASNLHTGVPSRFSGSGSGTDFTFTISSLQPEDIATYYCQQGQTYPLTFGGGTKVEIK

SEQ ID NO: 18 - protein, 11 aa, synthetic construct
HASQNINVWLS

SEQ ID NO: 19 - protein, 7 aa, synthetic construct
KASNLHT

SEQ ID NO: 20 - protein, 9 aa, synthetic construct
QQGQTYPLT

SEQ ID NO: 21 - protein, 330 aa, synthetic construct
ASTKGPSVFPLAPSSKSTSGGTAALGCLVKDYFPEPVTVSWNSGALTSGVHTFPAVLQSSGLYSLSSVVTVPSSSLGTQTYICNVNHKPSNTKVDKKVEPKSCDKTHTCPPCPAPEAAGGPSVFLFPPKPKDTLMISRTPEVTCVVVDVSHEDPEVKFNWYVDGVEVHNAKTKPREEQYNSTYRVVSVLTVLHQDWLNGKEYKCKVSNKALPAPIEKTISKAKGQPREPQVYTLPPSREEMTKNQVSLTCLVKGFYPSDIAVEWESNGQPENNYKTTPPVLDSDGSFFLYSKLTVDKSRWQQGNVFSCSVMHEALHNHYTQKSLSLSPGK

SEQ ID NO: 22 - protein, 107 aa, synthetic construct
RTVAAPSVFIFPPSDEQLKSGTASVVCLLNNFYPREAKVQWKVDNALQSGNSQESVTEQDSKDSTYSLSSTLTLSKADYEKHKVYACEVTHQGLSSPVTKSFNRGEA

SEQ ID NO: 23 - protein, 329 aa, synthetic construct
ASTKGPSVFPLAPSSKSTSGGTAALGCLVKDYFPEPVTVSWNSGALTSGVHTFPAVLQSSGLYSLSSVVTVPSSSLGTQTYICNVNHKPSNTKVDKKVEPKSCDKTHTCPPCPAPEAAGGPSVFLFPPKPKDTLMISRTPEVTCVVVDVSHEDPEVKFNWYVDGVEVHNAKTKPREEQYNSTYRVVSVLTVLHQDWLNGKEYKCKVSNKALPAPIEKTISKAKGQPREPQVYTLPPSREEMTKNQVSLTCLVKGFYPSDIAVEWESNGQPENNYKTTPPVLDSDGSFFLYSKLTVDKSRWQQGNVFSCSVMHEALHNHYTQKSLSLSPG

SEQ ID NO: 24 - protein, 582 aa, synthetic construct
EVQLVESGGGVVQPGRSLRLSCVASGFPFNNYWMTWIRQAPGKGLEWIASITITGGTTYYPGSVKGRFTISRDNSKSTLYLQMNSLRAEDTAVYYCTRERYSTEYYPYYWYFDFWGQGTMVTVSSGGGGSGGGGSEVQLVQSGAEVKKPGSSVKVSCKASGYTFTDYYMNWVKQAPGKGLEWIGLINPSNTGTNYNQKFRDKATLTVDKSTSTAYMELSSLRSEDTAVYYCARRAQATSGDYWGQGTTVTVSSASTKGPSVFPLAPSSKSTSGGTAALGCLVKDYFPEPVTVSWNSGALTSGVHTFPAVLQSSGLYSLSSVVTVPSSSLGTQTYICNVNHKPSNTKVDKKVEPKSCDKTHTCPPCPAPEAAGGPSVFLFPPKPKDTLMISRTPEVTCVVVDVSHEDPEVKFNWYVDGVEVHNAKTKPREEQYNSTYRVVSVLTVLHQDWLNGKEYKCKVSNKALPAPIEKTISKAKGQPREPQVYTLPPSREEMTKNQVSLTCLVKGFYPSDIAVEWESNGQPENNYKTTPPVLDSDGSFFLYSKLTVDKSRWQQGNVFSCSVMHEALHNHYTQKSLSLSPG

SEQ ID NO: 25 - protein, 6 aa, synthetic construct
GGGGSG

SEQ ID NO: 26 - protein, 14 aa, synthetic construct
GGGGSGGGGSGGGG

SEQ ID NO: 27 - protein, 5 aa, synthetic construct
GGSGG

SEQ ID NO: 28 - protein, 13 aa, synthetic construct
GGSGGGGSGGGGS